European Patent Specification EP 4 203 959 B1, published August 14, 2024. Title: Trabectedin for the treatment of cancer. Applicant: Anturec Pharmaceuticals GmbH. The sequence listing filed with the application follows.

SEQUENCE LISTING (2 sequences)

SEQ ID NO: 1 - protein, 225 aa, Artificial Sequence
  tTF-NGR fusion protein
SGTTNTVAAYNLTWKSTNFKTILEWEPKPVNQVYTVQISTKSGDWKSKCFYTTDTECDLTDEIVKDVKQTYLARVFSYPAGNVESTGSAGEPLYENSPEFTPYLETNLGQPTIQSFEQVGTKVNVTVEDERTLVRRNNTFLSLRDVFGKDLIYTLYYWKSSSSGKKTAKTNTNEFLIDVDKGENYCFSVQAVIPSRTVNRKSTDSPVECMGQEKGEFRGNGRAHA

SEQ ID NO: 2 - protein, 271 aa, Artificial Sequence
  His-tTF-NGR fusion protein
MHHHHHHSSGLVPRGSGMKETAAAKFERQHMDSPDLGTDDDDKAMGSGTTNTVAAYNLTWKSTNFKTILEWEPKPVNQVYTVQISTKSGDWKSKCFYTTDTECDLTDEIVKDVKQTYLARVFSYPAGNVESTGSAGEPLYENSPEFTPYLETNLGQPTIQSFEQVGTKVNVTVEDERTLVRRNNTFLSLRDVFGKDLIYTLYYWKSSSSGKKTAKTNTNEFLIDVDKGENYCFSVQAVIPSRTVNRKSTDSPVECMGQEKGEFRGNGRAHA